European Patent Application EP 4 261 283 A1, published October 18, 2023. Title: Compositions for treating or preventing muscle diseases, obesity or diabetes. Applicant: NUON BIO Co.,Ltd. The sequence listing filed with the application follows.

SEQUENCE LISTING (4 sequences)

SEQ ID NO: 1 - protein, 967 aa, Artificial Sequence
  ADAMTS1
MQRAVPEGFGRRKLGSDMGNAERAPGSRSFGPVPTLLLLAAALLAVSDALGRPSEEDEELVVPELERAPGHGTTRLRLHAFDQQLDLELRPDSSFLAPGFTLQNVGRKSGSETPLPETDLAHCFYSGTVNGDPSSAAALSLCEGVRGAFYLLGEAYFIQPLPAASERLATAAPGEKPPAPLQFHLLRRNRQGDVGGTCGVVDDEPRPTGKAETEDEDEGTEGEDEGAQWSPQDPALQGVGQPTGTGSIRKKRFVSSHRYVETMLVADQSMAEFHGSGLKHYLLTLFSVAARLYKHPSIRNSVSLVVVKILVIHDEQKGPEVTSNAALTLRNFCNWQKQHNPPSDRDAEHYDTAILFTRQDLCGSQTCDTLGMADVGTVCDPSRSCSVIEDDGLQAAFTTAHELGHVFNMPHDDAKQCASLNGVNQDSHMMASMLSNLDHSQPWSPCSAYMITSFLDNGHGECLMDKPQNPIQLPGDLPGTSYDANRQCQFTFGEDSKHCPDAASTCSTLWCTGTSGGVLVCQTKHFPWADGTSCGEGKWCINGKCVNKTDRKHFDTPFHGSWGMWGPWGDCSRTCGGGVQYTMRECDNPVPKNGGKYCEGKRVRYRSCNLEDCPDNNGKTFREEQCEAHNEFSKASFGSGPAVEWIPKYAGVSPKDRCKLICQAKGIGYFFVLQPKVVDGTPCSPDSTSVCVQGQCVKAGCDRIIDSKKKFDKCGVCGGNGSTCKKISGSVTSAKPGYHDIITIPTGATNIEVKQRNQRGSRNNGSFLAIKAADGTYILNGDYTLSTLEQDIMYKGVVLRYSGSSAALERIRSFSPLKEPLTIQVLTVGNALRPKIKYTYFVKKKKESFNAIPTFSAWVIEEWGECSKSCELGWQRRLVECRDINGQPASECAKEVKPASTRPCADHPCPQWQLGEWSSCSKTCGKGYKKRSLKCLSHDGGVLSHESCDPLKKPKHFIDFCTMAECS

SEQ ID NO: 2 - protein, 382 aa, Artificial Sequence
  M3
MQRAVPEGFGRRKLGSDMGNAERAPGSRSFGPVPTLLLLAAALLAVSDALGRPSEEDEELVVPELERAPGHGTTRLRLHAFDQQLDLELRPDSSFLAPGFTLQNVGRKSGSETPLPETDLAHCFYSGTVNGDPSSAAALSLCEGVRGAFYLLGEAYFIQPLPAASERLATAAPGEKPPAPLQFHLLRRNRQGDVGGTCGVVDDEPRPTGKAETEDEDEGTERFVSSHRYVETMLVADQSMAEFHGSGLKHYLLTLFSVAARLYKHPSIRNSVSLVVVKILVIHDEQKGPEVTSNAALTLRNFCNWQKQHNPPSDRDAEHYDTAILFTRQDLCGSQTCDTLGMADVGTVCDPSRSCSVIEDDGLQAAFTTAHELGHVFNMPHD

SEQ ID NO: 3 - DNA, 2904 bp, Artificial Sequence
  ADAMTS1
atgcagcgagctgtgcccgaggggttcggaaggcgcaagctgggcagcgacatggggaacgcggagcgggctccggggtctcggagctttgggccagtacccacgctgctgctgctcgccgcggcgctactggccgtgtcggacgcactcgggcgcccctccgaggaggacgaggagctagtggtgccggagctggagcgcgccccgggacacgggaccacgcgcctccgcctgcacgcctttgaccagcagctggatctggagctgcggcccgacagcagctttttggcgcccggcttcacgctccagaacgtggggcgcaaatccgggtccgagacgccgcttccggaaaccgacctggcgcactgcttctactccggcaccgtgaatggcgatcccagctcggctgccgccctcagcctctgcgagggcgtgcgcggcgccttctacctgctgggggaggcgtatttcatccagccgctgcccgccgccagcgagcgcctcgccaccgccgccccaggggagaagccgccggcaccactacagttccacctcctgcggcggaatcggcagggcgacgtcggcggcacgtgcggggtcgtggacgacgagccccggccgactgggaaagcggagaccgaagacgaggacgaagggactgagggcgaggacgaaggggctcagtggtcgccgcaggacccggcactgcaaggcgtaggacagcccacaggaactggaagcataagaaagaagcgatttgtgtccagtcaccgctatgtggaaaccatgcttgtggcagaccagtcgatggcagaattccacggcagtggtctaaagcattaccttctcacgttgttttcggtggcagccagattgtacaaacaccccagcattcgtaattcagttagcctggtggtggtgaagatcttggtcatccacgatgaacagaaggggccggaagtgacctccaatgctgccctcactctgcggaacttttgcaactggcagaagcagcacaacccacccagtgaccgggatgcagagcactatgacacagcaattcttttcaccagacaggacttgtgtgggtcccagacatgtgatactcttgggatggctgatgttggaactgtgtgtgatccgagcagaagctgctccgtcatagaagatgatggtttacaagctgccttcaccacagcccatgaattaggccacgtgtttaacatgccacatgatgatgcaaagcagtgtgccagccttaatggtgtgaaccaggattcccacatgatggcgtcaatgctttccaacctggaccacagccagccttggtctccttgcagtgcctacatgattacatcatttctggataatggtcatggggaatgtttgatggacaagcctcagaatcccatacagctcccaggcgatctccctggcacctcgtacgatgccaaccggcagtgccagtttacatttggggaggactccaaacactgccccgatgcagccagcacatgtagcaccttgtggtgtaccggcacctctggtggggtgctggtgtgtcaaaccaaacacttcccgtgggcggatggcaccagctgtggagaagggaaatggtgtatcaacggcaagtgtgtgaacaaaaccgacagaaagcattttgatacgccttttcatggaagctggggaatgtgggggccttggggagactgttcgagaacgtgcggtggaggagtccagtacacgatgagggaatgtgacaacccagtcccaaagaatggagggaagtactgtgaaggcaaacgagtgcgctacagatcctgtaaccttgaggactgtccagacaataatggaaaaacctttagagaggaacaatgtgaagcacacaacgagttttcaaaagcttcctttgggagtgggcctgcggtggaatggattcccaagtacgctggcgtctcaccaaaggacaggtgcaagctcatctgccaagccaaaggcattggctacttcttcgttttgcagcccaaggttgtagatggtactccatgtagcccagattccacctctgtctgtgtgcaaggacagtgtgtaaaagctggttgtgatcgcatcatagactccaaaaagaagtttgataaatgtggtgtttgcgggggaaatggatctacttgtaaaaaaatatcaggatcagttactagtgcaaaacctggatatcatgatatcatcacaattccaactggagccaccaacatcgaagtgaaacagcggaaccagaggggatccaggaacaatggcagctttcttgccatcaaagctgctgatggcacatatattcttaatggtgactacactttgtccaccttagagcaagacattatgtacaaaggtgttgtcttgaggtacagcggctcctctgcggcattggaaagaattcgcagctttagccctctcaaagagcccttgaccatccaggttcttactgtgggcaatgcccttcgacctaaaattaaatacacctacttcgtaaagaagaagaaggaatctttcaatgctatccccactttttcagcatgggtcattgaagagtggggcgaatgttctaagtcatgtgaattgggttggcagagaagactggtagaatgccgagacattaatggacagcctgcttccgagtgtgcaaaggaagtgaagccagccagcaccagaccttgtgcagaccatccctgcccccagtggcagctgggggagtggtcatcatgttctaagacctgtgggaagggttacaaaaaaagaagcttgaagtgtctgtcccatgatggaggggtgttatctcatgagagctgtgatcctttaaagaaacctaaacatttcatagacttttgcacaatggcagaatgcagttaa

SEQ ID NO: 4 - DNA, 1146 bp, Artificial Sequence
  M3
atgcagcgagctgtgcccgaggggttcggaaggcgcaagctgggcagcgacatggggaacgcggagcgggctccggggtctcggagctttgggccagtacccacgctgctgctgctcgccgcggcgctactggccgtgtcggacgcactcgggcgcccctccgaggaggacgaggagctagtggtgccggagctggagcgcgccccgggacacgggaccacgcgcctccgcctgcacgcctttgaccagcagctggatctggagctgcggcccgacagcagctttttggcgcccggcttcacgctccagaacgtggggcgcaaatccgggtccgagacgccgcttccggaaaccgacctggcgcactgcttctactccggcaccgtgaatggcgatcccagctcggctgccgccctcagcctctgcgagggcgtgcgcggcgccttctacctgctgggggaggcgtatttcatccagccgctgcccgccgccagcgagcgcctcgccaccgccgccccaggggagaagccgccggcaccactacagttccacctcctgcggcggaatcggcagggcgacgtcggcggcacgtgcggggtcgtggacgacgagccccggccgactgggaaagcggagaccgaagacgaggacgaagggactgagcgatttgtgtccagtcaccgctatgtggaaaccatgcttgtggcagaccagtcgatggcagaattccacggcagtggtctaaagcattaccttctcacgttgttttcggtggcagccagattgtacaaacaccccagcattcgtaattcagttagcctggtggtggtgaagatcttggtcatccacgatgaacagaaggggccggaagtgacctccaatgctgccctcactctgcggaacttttgcaactggcagaagcagcacaacccacccagtgaccgggatgcagagcactatgacacagcaattcttttcaccagacaggacttgtgtgggtcccagacatgtgatactcttgggatggctgatgttggaactgtgtgtgatccgagcagaagctgctccgtcatagaagatgatggtttacaagctgccttcaccacagcccatgaattaggccacgtgtttaacatgccacatgat